European Patent Specification EP 3 729 101 B1, published March 18, 2026. Title: WORKFLOW FOR RISK ASSESSMENT AND PATIENT MANAGEMENT USING. Applicant: B.R.A.H.M.S GmbH. Application EP17209151.4. The sequence listing filed with the application follows.

SEQUENCE LISTING (4 sequences)

SEQ ID NO: 1 - protein, 116 aa, Homo sapiens
APFRSALESSPADPATLSEDEARLLLAALVQDYVQMKASELEQEQEREGSSLDSPRSKRCGNLSTCMLGTYTQDFNKFHTFPQTAIGVGAPGKKRDMSSDLERDHRPHVSMPQNAN

SEQ ID NO: 2 - protein, 48 aa, Homo sapiens
ELRMSSSYPTGLADVKAGPAQTLIRPQDMKGASRSPEDSSPDAARIRV

SEQ ID NO: 3 - protein, 164 aa, Homo sapiens
ARLDVASEFRKKWNKWALSRGKRELRMSSSYPTGLADVKAGPAQTLIRPQDMKGASRSPEDSSPDAARIRVKRYRQSMNNFQGLRSFGCRFGTCTVQKLAHQIYQFTDKDKDNVAPRSKISPQGYGRRRRRSLPEAGPGRTLVSSKPQAHGAPAPPSGSAPHFL

SEQ ID NO: 4 - protein, 185 aa, Homo sapiens
MKLVSVALMYLGSLAFLGADTARLDVASEFRKKWNKWALSRGKRELRMSSSYPTGLADVKAGPAQTLIRPQDMKGASRSPEDSSPDAARIRVKRYRQSMNNFQGLRSFGCRFGTCTVQKLAHQIYQFTDKDKDNVAPRSKISPQGYGRRRRRSLPEAGPGRTLVSSKPQAHGAPAPPSGSAPHFL